European Patent Application EP 4 537 845 A1, published April 16, 2025. Title: ＴｙｐｅＩ味覚受容体（Ｔ１Ｒｓ）を介した膜電位依存性イオンチャネルの制御方法. Applicant: 株式会社　Ion Chat Research. Application JP. The sequence listing filed with the application follows.

SEQUENCE LISTING (7 sequences)

SEQ ID NO: 1 - protein, 11 aa, Homo sapiens
  source 1..11: note = Amyloid beta peptide 25-35 aa region
GSNKGAIIGLM

SEQ ID NO: 2 - protein, 38 aa, Homo sapiens
  source 1..38: note = Amyloid beta peptide 1-38 aa region
DAEFRHDSGYEVHHQKLVFFAEDVGSNKGAIIGLMVGG

SEQ ID NO: 3 - protein, 40 aa, Homo sapiens
  source 1..40: note = Amyloid beta peptide 1-40 aa region
DAEFRHDSGYEVHHQKLVFFAEDVGSNKGAIIGLMVGGVV

SEQ ID NO: 4 - protein, 42 aa, Homo sapiens [sequence omitted]

SEQ ID NO: 5 - protein, 30 aa, Homo sapiens
  source 1..30: note = Human T1R3 protein 229-258 aa region, Ligand binding domain as Venus Flytrap Domain region (LB2)
LAAARGICIAHEGLVPLPRADDSRLGKVQD

SEQ ID NO: 6 - protein, 94 aa, Homo sapiens
  source 1..94: note = Human T1R3 protein 303-396 aa region, Ligand binding site (LB1)
WLTSDLVMGLPGMAQMGTVLGFLQRGAQLHEFPQYVKTHLALATDPAFCSALGEREQGLEEDVVGQRCPQCDCITLQNVSAGLNHHQTFSVYAA

SEQ ID NO: 7 - protein, 201 aa, Homo sapiens
  source 1..201: note = Human T1R3 protein 400-570 aa region, Ligand binding site having Cysteine Rich Domain
VAQALHNTLQCNASGCPAQDPVKPWQLLENMYNLTFHVGGLPLRFDSSGNVDMEYDLKLWVWQGSVPRLHDVGRFNGSLRTERLKIRWHTSDNQKPVSRCSRQCQEGQVRRVKGFHSCCYDCVDCEAGSYRQNPDDIACTFCGQDEWSPERSTRCFRRRSRFLAWGEPAVLLLLLLLSLALGLVLAALGLFVHHRDSPLVQ